European Patent Application EP 4 803 548 A1, published September 9, 2026. Title: 结合HLA-A02/HBsAg复合体的多种抗体及其用途. Applicant: 北京智仁美博生物科技有限公司. The sequence listing filed with the application follows.

SEQUENCE LISTING (88 sequences)

SEQ ID NO: 1 - protein, 10 aa, homo sapiens
GLSPTVWLSV

SEQ ID NO: 2 - protein, 10 aa, homo sapiens
GLSPTVWLSV

SEQ ID NO: 3 - protein, 10 aa, homo sapiens
KLLEPVPVSV

SEQ ID NO: 4 - protein, 10 aa, homo sapiens
GLWHGILTSV

SEQ ID NO: 5 - protein, 10 aa, homo sapiens
GLVGNPLPSV

SEQ ID NO: 6 - protein, 10 aa, homo sapiens
VLEDGPWKTV

SEQ ID NO: 7 - protein, 10 aa, homo sapiens
FLPQPVPLSV

SEQ ID NO: 8 - protein, 10 aa, homo sapiens
FLPQPVPLSV

SEQ ID NO: 9 - protein, 10 aa, homo sapiens
GLINTGVLSV

SEQ ID NO: 10 - protein, 10 aa, homo sapiens
ALSPITKLSV

SEQ ID NO: 11 - protein, 10 aa, homo sapiens
GLSPLRPPSV

SEQ ID NO: 12 - protein, 10 aa, homo sapiens
GLSEEKPLSV

SEQ ID NO: 13 - protein, 10 aa, homo sapiens
GLSPVTNLTV

SEQ ID NO: 14 - protein, 10 aa, homo sapiens
SGLSPTVAVL

SEQ ID NO: 15 - protein, 9 aa, homo sapiens
SLSPTVWFL

SEQ ID NO: 16 - protein, 9 aa, homo sapiens
AQPTVWLTI

SEQ ID NO: 17 - protein, 10 aa, homo sapiens
HLLSTPWLQL

SEQ ID NO: 18 - protein, 9 aa, homo sapiens
ILVDTVWAL

SEQ ID NO: 19 - protein, 9 aa, homo sapiens
KLLETKWTL

SEQ ID NO: 20 - protein, 10 aa, homo sapiens
RVPDFYFHTI

SEQ ID NO: 21 - protein, 10 aa, homo sapiens
SLAETFWETT

SEQ ID NO: 22 - protein, 10 aa, homo sapiens
YLPHTFWITL

SEQ ID NO: 23 - protein, 10 aa, homo sapiens
GLWHGVLTSV

SEQ ID NO: 24 - protein, 10 aa, homo sapiens
SLAERLFFQV

SEQ ID NO: 25 - protein, 10 aa, homo sapiens
WLQDFVPTSV

SEQ ID NO: 26 - protein, 10 aa, homo sapiens
WLLPGRWTSV

SEQ ID NO: 27 - protein, 10 aa, homo sapiens
LLLATVLQAV

SEQ ID NO: 28 - protein, 10 aa, homo sapiens
YLKDGPYITA

SEQ ID NO: 29 - protein, 9 aa, homo sapiens
GLMDTVKKV

SEQ ID NO: 30 - protein, 10 aa, homo sapiens
ALDSGAFQSV

SEQ ID NO: 31 - protein, 10 aa, homo sapiens
FLWDEGFHQL

SEQ ID NO: 32 - protein, 5 aa, Camelus
TNCMG

SEQ ID NO: 33 - protein, 17 aa, Camelus
AIYTGGGRAVYADSVRG

SEQ ID NO: 34 - protein, 21 aa, Camelus
DWLGPDMTDIQVLGALPWFNY

SEQ ID NO: 35 - protein, 130 aa, Camelus
QVQLVESGGGSVQAGGSLRLSCAASDDTYMTNCMGWFRQAPGKEREGVAAIYTGGGRAVYADSVRGRFTISQDNAKNTVYLQMNSLKPEDTAMYYCAADWLGPDMTDIQVLGALPWFNYWGQGTLVTVSS

SEQ ID NO: 36 - protein, 130 aa, synthetic construct
EVQLVESGGGLVQPGGSLRLSCAASDDTYMTNCMGWFRQAPGKERVGVAAIYTGGGRAVYADSVRGRFTISQDNAKNTVYLQMNSLKPEDTAMYYCAADWLGPDMTDIQVLGALPWFNYWGQGTLVTVSS

SEQ ID NO: 37 - protein, 5 aa, synthetic construct
GYTMN

SEQ ID NO: 38 - protein, 17 aa, synthetic construct
LINPYKGVSTYNQKFKD

SEQ ID NO: 39 - protein, 13 aa, synthetic construct
SGYYGDSDWYFDV

SEQ ID NO: 40 - protein, 11 aa, synthetic construct
RASQDIRNYLN

SEQ ID NO: 41 - protein, 7 aa, synthetic construct
YTSRLES

SEQ ID NO: 42 - protein, 9 aa, synthetic construct
QQGNTLPWT

SEQ ID NO: 43 - protein, 122 aa, synthetic construct [sequence omitted]

SEQ ID NO: 44 - protein, 107 aa, synthetic construct [sequence omitted]

SEQ ID NO: 45 - protein, 506 aa, synthetic construct
QVQLVESGGGSVQAGGSLRLSCAASDDTYMTNCMGWFRQAPGKEREGVAAIYTGGGRAVYADSVRGRFTISQDNAKNTVYLQMNSLKPEDTAMYYCAADWLGPDMTDIQVLGALPWFNYWGQGTLVTVSSGGGGSGGGGSGGGGSQVQLVESGGGSVQAGGSLRLSCAASDDTYMTNCMGWFRQAPGKEREGVAAIYTGGGRAVYADSVRGRFTISQDNAKNTVYLQMNSLKPEDTAMYYCAADWLGPDMTDIQVLGALPWFNYWGQGTLVTVSSASERKSSVECPPCPAPEFEGGPSVFLFPPKPKDTLMISRTPEVTCVVVDVSQEDPEVQFNWYVDGVEVHNAKTKPREEQYNSTYRVVSVLTVLHQDWLNGKEYKCKVSNKALPASIEKTISKAKGQPREPQVCTLPPSQEEMTKNQVSLSCAVKGFYPSDIAVEWESNGQPENNYKTTPPVLDSDGSFFLVSKLTVDKSRWQEGNVFSCSVMHEALHNHYTQKSLSLSPGK

SEQ ID NO: 46 - protein, 506 aa, synthetic construct
EVQLVESGGGLVQPGGSLRLSCAASDDTYMTNCMGWFRQAPGKERVGVAAIYTGGGRAVYADSVRGRFTISQDNAKNTVYLQMNSLKPEDTAMYYCAADWLGPDMTDIQVLGALPWFNYWGQGTLVTVSSGGGGSGGGGSGGGGSEVQLVESGGGLVQPGGSLRLSCAASDDTYMTNCMGWFRQAPGKERVGVAAIYTGGGRAVYADSVRGRFTISQDNAKNTVYLQMNSLKPEDTAMYYCAADWLGPDMTDIQVLGALPWFNYWGQGTLVTVSSASERKSSVECPPCPAPEFEGGPSVFLFPPKPKDTLMISRTPEVTCVVVDVSQEDPEVQFNWYVDGVEVHNAKTKPREEQYNSTYRVVSVLTVLHQDWLNGKEYKCKVSNKALPASIEKTISKAKGQPREPQVCTLPPSQEEMTKNQVSLSCAVKGFYPSDIAVEWESNGQPENNYKTTPPVLDSDGSFFLVSKLTVDKSRWQEGNVFSCSVMHEALHNHYTQKSLSLSPGK

SEQ ID NO: 47 - protein, 484 aa, synthetic construct
DIQMTQSPSSLSASVGDRVTITCRASQDIRNYLNWYQQKPGKAPKLLIYYTSRLESGVPSRFSGSGSGTDYTLTISSLQPEDFATYYCQQGNTLPWTFGQGTKVEIKGGGGSGGGGSGGGGSGGGGSGGGSEVQLVESGGGLVQPGGSLRLSCAASGYSFTGYTMNWVRQAPGKGLEWVALINPYKGVSTYNQKFKDRFTISVDKSKNTAYLQMNSLRAEDTAVYYCARSGYYGDSDWYFDVWGQGTLVTVSSASERKSSVECPPCPAPEFEGGPSVFLFPPKPKDTLMISRTPEVTCVVVDVSHEDPEVKFNWYVDGVEVHNAKTKPREEQYNSTYRVVSVLTVLHQDWLNGKEYKCKVSNKALPASIEKTISKAKGQPREPQVYTLPPCREEMTKNQVSLWCLVKGFYPSDIAVEWESNGQPENNYKTTPPVLDSDGSFFLYSKLTVDKSRWQQGNVFSCSVMHEALHNHYTQKSLSLSPGK

SEQ ID NO: 48 - protein, 105 aa, homo sapiens
QDGNEEMGGITQTPYKVSISGTTVILTCPQYPGSEILWQHNDKNIGGDEDDKNIGSDEDHLSLKEFSELEQSGYYVCYPRGSKPEDANFYLYLRARVCENCMEMD

SEQ ID NO: 49 - protein, 84 aa, homo sapiens [sequence omitted]

SEQ ID NO: 50 - protein, 419 aa, synthetic construct
GLSPTVWLSVGCGGSGGGGSGGGGSIQRTPKIQVYSRHPAENGKSNFLNCYVSGFHPSDIEVDLLKNGERIEKVEHSDLSFSKDWSFYLLYYTEFTPTEKDEYACRVNHVTLSQPKIVKWDRDMGGGGSGGGGSGGGGSGGGGSGSHSMRYFFTSVSRPGRGEPRFIAVGYVDDTQFVRFDSDAASQRMEPRAPWIEQEGPEYWDGETRKVKAHSQTHRVDLGTLRGCYNQSEAGSHTVQRMYGCDVGSDWRFLRGYHQYAYDGKDYIALKEDLRSWTAADMAAQTTKHKWEAAHVAEQLRAYLEGTCVEWLRRYLENGKETLQRTDAPKTHMTHHAVSDHEATLRCWALSFYPAEITLTWQRDGEDQTQDTELVETRPAGDGTFQKWAAVVVPSGQEQRYTCHVQHEGLPKPLTLRWE

SEQ ID NO: 51 - protein, 389 aa, synthetic construct
MGTNLSVPNPLGFFPDHQLDPAFGANSNNPDWDFNPNKDQWPEANQVGAGAFGPGFTPPHGGLLGWSPQAQGILTTVPAAPPPASTNRQSGRQPTPISPPLRDSHPQAMQWNSTTFHQALLDPRVRGLYFPAGGSSSGTVNPVPTIVSPISSIFSRTGDPAPNMESTTSGFLGPLLVLQAGFFLLTRILTIPQSLDSWWTSLNFLGEAPTCPGQNSQSPTSNHSPTSCPPICPGYRWMCLRRFIIFLFILLLCLIFLLVLLDYQGMLPVCPLLPGTSTTSTGPCKTCTIPAQGTSMFPSCCCTKPSDGNCTCIPIPSSWAFARFLWEWASVRFSWLSLLVPFVQWFAGLSPTVWLSVIWMMWYWGPSLYNILSPFLPLLPIFFCLWVYI

SEQ ID NO: 52 - protein, 15 aa, synthetic construct
GGGGSGGGGSGGGGS

SEQ ID NO: 53 - DNA, 22 bp, synthetic construct
  source 1..22: mol_type = other DNA
tccttccccgtcagccagtcct

SEQ ID NO: 54 - protein, 6 aa, synthetic construct
HHHHHH

SEQ ID NO: 55 - protein, 234 aa, mus musculus
ASPRGPTIKPCPPCKCPAPNLLGGPSVFIFPPKIKDVLMISLSPIVTCVVVDVSEDDPDVQISWFVNNVEVHTAQTQTHREDYNSTLRVVSALPIQHQDWMSGKEFKCKVNNKDLPAPIERTISKPKGSVRAPQVYVLPPPEEEMTKKQVTLTCMVTDFMPEDIYVEWTNNGKTELNYKNTEPVLDSDGSYFMYSKLRVEKKNWVERNSYSCSVVHEGLHNHHTTKSFSRTPGK

SEQ ID NO: 56 - protein, 330 aa, homo sapiens
ASTKGPSVFPLAPSSKSTSGGTAALGCLVKDYFPEPVTVSWNSGALTSGVHTFPAVLQSSGLYSLSSVVTVPSSSLGTQTYICNVNHKPSNTKVDKRVEPKSCDKTHTCPPCPAPELLGGPSVFLFPPKPKDTLMISRTPEVTCVVVDVSHEDPEVKFNWYVDGVEVHNAKTKPREEQYNSTYRVVSVLTVLHQDWLNGKEYKCKVSNKALPAPIEKTISKAKGQPREPQVYTLPPSREEMTKNQVSLTCLVKGFYPSDIAVEWESNGQPENNYKTTPPVLDSDGSFFLYSKLTVDKSRWQQGNVFSCSVMHEALHNHYTQKSLSLSPGK

SEQ ID NO: 57 - protein, 330 aa, synthetic construct
ASTKGPSVFPLAPSSKSTSGGTAALGCLVKDYFPEPVTVSWNSGALTSGVHTFPAVLQSSGLYSLSSVVTVPSSSLGTQTYICNVNHKPSNTKVDKRVEPKSCDKTHTCPPCPAPELLGGPSVFLFPPKPKDTLMISRTPEVTCVVVDVSHEDPEVKFNWYVDGVEVHNAKTKPREEQYNSTYRVVSVLTVLHQDWLNGKEYKCKVSNKALPAPIEKTISKAKGQPREPQVCTLPPSREEMTKNQVSLSCAVKGFYPSDIAVEWESNGQPENNYKTTPPVLDSDGSFFLVSKLTVDKSRWQQGNVFSCSVMHEALHNHYTQKSLSLSPGK

SEQ ID NO: 58 - protein, 330 aa, synthetic construct
ASTKGPSVFPLAPSSKSTSGGTAALGCLVKDYFPEPVTVSWNSGALTSGVHTFPAVLQSSGLYSLSSVVTVPSSSLGTQTYICNVNHKPSNTKVDKRVEPKSCDKTHTCPPCPAPELLGGPSVFLFPPKPKDTLMISRTPEVTCVVVDVSHEDPEVKFNWYVDGVEVHNAKTKPREEQYNSTYRVVSVLTVLHQDWLNGKEYKCKVSNKALPAPIEKTISKAKGQPREPQVYTLPPCREEMTKNQVSLWCLVKGFYPSDIAVEWESNGQPENNYKTTPPVLDSDGSFFLYSKLTVDKSRWQQGNVFSCSVMHEALHNHYTQKSLSLSPGK

SEQ ID NO: 59 - protein, 330 aa, synthetic construct
ASTKGPSVFPLAPSSKSTSGGTAALGCLVKDYFPEPVTVSWNSGALTSGVHTFPAVLQSSGLYSLSSVVTVPSSSLGTQTYICNVNHKPSNTKVDKRVEPKSCDKTHTCPPCPAPEFEGGPSVFLFPPKPKDTLMISRTPEVTCVVVDVSHEDPEVKFNWYVDGVEVHNAKTKPREEQYNSTYRVVSVLTVLHQDWLNGKEYKCKVSNKALPASIEKTISKAKGQPREPQVCTLPPSREEMTKNQVSLSCAVKGFYPSDIAVEWESNGQPENNYKTTPPVLDSDGSFFLVSKLTVDKSRWQQGNVFSCSVMHEALHNHYTQKSLSLSPGK

SEQ ID NO: 60 - protein, 330 aa, synthetic construct
ASTKGPSVFPLAPSSKSTSGGTAALGCLVKDYFPEPVTVSWNSGALTSGVHTFPAVLQSSGLYSLSSVVTVPSSSLGTQTYICNVNHKPSNTKVDKRVEPKSCDKTHTCPPCPAPEFEGGPSVFLFPPKPKDTLMISRTPEVTCVVVDVSHEDPEVKFNWYVDGVEVHNAKTKPREEQYNSTYRVVSVLTVLHQDWLNGKEYKCKVSNKALPASIEKTISKAKGQPREPQVYTLPPCREEMTKNQVSLWCLVKGFYPSDIAVEWESNGQPENNYKTTPPVLDSDGSFFLYSKLTVDKSRWQQGNVFSCSVMHEALHNHYTQKSLSLSPGK

SEQ ID NO: 61 - protein, 327 aa, synthetic construct
ASTKGPSVFPLAPSSKSTSEGTAALGCLVKDYFPEPVTVSWNSGALTSGVHTFPAVLQSSGLYSLSSVVTVPSSSLGTQTYICNVDHKPSNTKVDKTVERKSCVECPPCPAPEFEGGPSVFLFPPKPKDTLMISRTPEVTCVVVDVSQEDPEVQFNWYVDGVEVHNAKTKPREEQYNSTYRVVSVLTVLHQDWLNGKEYKCKVSNKALPASIEKTISKAKGQPREPQVCTLPPSQEEMTKNQVSLSCAVKGFYPSDIAVEWESNGQPENNYKTTPPVLDSDGSFFLVSKLTVDKSRWQEGNVFSCSVMHEALHNHYTQKSLSLSPGK

SEQ ID NO: 62 - protein, 327 aa, synthetic construct
ASTKGPSVFPLAPSSKSTSGGTAALGCLVKDYFPEPVTVSWNSGALTSGVHTFPAVLQSSGLYSLSSVVTVPSSSLGTQTYICNVNHKPSNTKVDKRVERKSCVECPPCPAPEFEGGPSVFLFPPKPKDTLMISRTPEVTCVVVDVSHEDPEVKFNWYVDGVEVHNAKTKPREEQYNSTYRVVSVLTVLHQDWLNGKEYKCKVSNKALPASIEKTISKAKGQPREPQVYTLPPCREEMTKNQVSLWCLVKGFYPSDIAVEWESNGQPENNYKTTPPVLDSDGSFFLYSKLTVDKSRWQQGNVFSCSVMHEALHNHYTQKSLSLSPGK

SEQ ID NO: 63 - protein, 106 aa, homo sapiens
GQPKAAPSVTLFPPSSEELQANKATLVCLISDFYPGAVTVAWKADSSPVKAGVETTTPSKQSNNKYAASSYLSLTPEQWKSHRSYSCQVTHEGSTVEKTVAPTECS

SEQ ID NO: 64 - protein, 107 aa, homo sapiens [sequence omitted]

SEQ ID NO: 65 - protein, 115 aa, synthetic construct
EVQLLESGGGLVQPGGSLRLSCAASGFTFSSYAMSWVRQAPGKGLEWVSAISGSGGSTYYADSVKGRFTISRDNSKNTLYLQMNSLRAEDTAVYYCAKGSGFDYWGQGTLVTVSS

SEQ ID NO: 66 - protein, 108 aa, synthetic construct
EIVLTQSPGTLSLSPGERATLSCRASQSVSSSYLAWYQQKPGQAPRLLIYGASSRATGIPDRFSGSGSGTDFTLTISRLEPEDFAVYYCQQYGSSPLTFGQGTKVEIK

SEQ ID NO: 67 - protein, 111 aa, synthetic construct
AKEVEQNSGPLSVPEGAIASLNCTYSDRGSQSFFWYRQYSGKGPELIMSIYSDGDKEDGRFTAQLNKASQYVSLLIRDSQPSDSATYLCAARNYKTDLLIFGTGTRLQVFP

SEQ ID NO: 68 - protein, 114 aa, synthetic construct
NAGVTQTPKFQVLKTGQSMTLQCAQDMSHGYMSWYRQDPGMGLRLIHYSVGAGITDQGEVPNGYNVSRSTTEDFPLRLLSAAPSQTSVYFCASSYATGGTGDLFFGEGSRLTVL

SEQ ID NO: 69 - protein, 442 aa, synthetic construct
AKEVEQNSGPLSVPEGAIASLNCTYSDRGSQSFFWYRQYSGKGPELIMSIYSDGDKEDGRFTAQLNKASQYVSLLIRDSQPSDSATYLCAARNYKTDLLIFGTGTRLQVFPYIQNPDPAVYQLRDSKSSDKFVCLFTDFDSQINVSQSKDSDVYITDKCVLDMRSMDFKSNSAVAWSNKSDFTCANAFNNSIIPEDTFFPSPESSCGGGGSASERKSSVECPPCPAPEFEGGPSVFLFPPKPKDTLMISRTPEVTCVVVDVSHEDPEVKFNWYVDGVEVHNAKTKPREEQYNSTYRVVSVLTVLHQDWLNGKEYKCKVSNKALPASIEKTISKAKGQPREPQVYTLPPCREEMTKNQVSLWCLVKGFYPSDIAVEWESNGQPENNYKTTPPVLDSDGSFFLYSKLTVDKSRWQQGNVFSCSVMHEALHNHYTQKSLSLSPGK

SEQ ID NO: 70 - protein, 481 aa, synthetic construct
NAGVTQTPKFQVLKTGQSMTLQCAQDMSHGYMSWYRQDPGMGLRLIHYSVGAGITDQGEVPNGYNVSRSTTEDFPLRLLSAAPSQTSVYFCASSYATGGTGDLFFGEGSRLTVLEDLKNVFPPEVAVFEPSKAEISRTQKATLVCLATGFYPPHVELSWWVNGKEVHDGVCTDPQPLKEQPALNDSRYALSSRLRVSATFWQDPRNHFRCQVQFYGLSENDEWTQDRAKPVTQIVSAEAWGRADCGGGGSASERKSCVECPPCPAPEFEGGPSVFLFPPKPKDTLMISRTPEVTCVVVDVSQEDPEVQFNWYVDGVEVHNAKTKPREEQYNSTYRVVSVLTVLHQDWLNGKEYKCKVSNKALPASIEKTISKAKGQPREPQVCTLPPSQEEMTKNQVSLSCAVKGFYPSDIAVEWESNGQPENNYKTTPPVLDSDGSFFLVSKLTVDKSRWQEGNVFSCSVMHEALHNHYTQKSLSLSPGK

SEQ ID NO: 71 - protein, 275 aa, synthetic construct
QVQLVESGGGSVQAGGSLRLSCAASDDTYMTNCMGWFRQAPGKEREGVAAIYTGGGRAVYADSVRGRFTISQDNAKNTVYLQMNSLKPEDTAMYYCAADWLGPDMTDIQVLGALPWFNYWGQGTLVTVSSGGGGSGGGGSGGGGSQVQLVESGGGSVQAGGSLRLSCAASDDTYMTNCMGWFRQAPGKEREGVAAIYTGGGRAVYADSVRGRFTISQDNAKNTVYLQMNSLKPEDTAMYYCAADWLGPDMTDIQVLGALPWFNYWGQGTLVTVSS

SEQ ID NO: 72 - protein, 275 aa, synthetic construct
EVQLVESGGGLVQPGGSLRLSCAASDDTYMTNCMGWFRQAPGKERVGVAAIYTGGGRAVYADSVRGRFTISQDNAKNTVYLQMNSLKPEDTAMYYCAADWLGPDMTDIQVLGALPWFNYWGQGTLVTVSSGGGGSGGGGSGGGGSEVQLVESGGGLVQPGGSLRLSCAASDDTYMTNCMGWFRQAPGKERVGVAAIYTGGGRAVYADSVRGRFTISQDNAKNTVYLQMNSLKPEDTAMYYCAADWLGPDMTDIQVLGALPWFNYWGQGTLVTVSS

SEQ ID NO: 73 - protein, 231 aa, synthetic construct
ASERKSSVECPPCPAPEFEGGPSVFLFPPKPKDTLMISRTPEVTCVVVDVSQEDPEVQFNWYVDGVEVHNAKTKPREEQYNSTYRVVSVLTVLHQDWLNGKEYKCKVSNKALPASIEKTISKAKGQPREPQVCTLPPSQEEMTKNQVSLSCAVKGFYPSDIAVEWESNGQPENNYKTTPPVLDSDGSFFLVSKLTVDKSRWQEGNVFSCSVMHEALHNHYTQKSLSLSPGK

SEQ ID NO: 74 - protein, 253 aa, synthetic construct
DIQMTQSPSSLSASVGDRVTITCRASQDIRNYLNWYQQKPGKAPKLLIYYTSRLESGVPSRFSGSGSGTDYTLTISSLQPEDFATYYCQQGNTLPWTFGQGTKVEIKGGGGSGGGGSGGGGSGGGGSGGGSEVQLVESGGGLVQPGGSLRLSCAASGYSFTGYTMNWVRQAPGKGLEWVALINPYKGVSTYNQKFKDRFTISVDKSKNTAYLQMNSLRAEDTAVYYCARSGYYGDSDWYFDVWGQGTLVTVSS

SEQ ID NO: 75 - protein, 231 aa, synthetic construct
ASERKSSVECPPCPAPEFEGGPSVFLFPPKPKDTLMISRTPEVTCVVVDVSHEDPEVKFNWYVDGVEVHNAKTKPREEQYNSTYRVVSVLTVLHQDWLNGKEYKCKVSNKALPASIEKTISKAKGQPREPQVYTLPPCREEMTKNQVSLWCLVKGFYPSDIAVEWESNGQPENNYKTTPPVLDSDGSFFLYSKLTVDKSRWQQGNVFSCSVMHEALHNHYTQKSLSLSPGK

SEQ ID NO: 76 - protein, 739 aa, synthetic construct
DIQMTQSPSSLSASVGDRVTITCRASQDIRNYLNWYQQKPGKAPKLLIYYTSRLESGVPSRFSGSGSGTDYTLTISSLQPEDFATYYCQQGNTLPWTFGQGTKVEIKGGGGSGGGGSGGGGSGGGGSGGGSEVQLVESGGGLVQPGGSLRLSCAASGYSFTGYTMNWVRQAPGKGLEWVALINPYKGVSTYNQKFKDRFTISVDKSKNTAYLQMNSLRAEDTAVYYCARSGYYGDSDWYFDVWGQGTLVTVSSGGGGSNAGVTQTPKFQVLKTGQSMTLQCAQDMSHGYMSWYRQDPGMGLRLIHYSVGAGITDQGEVPNGYNVSRSTTEDFPLRLLSAAPSQTSVYFCASSYATGGTGDLFFGEGSRLTVLEDLKNVFPPEVAVFEPSKAEISRTQKATLVCLATGFYPPHVELSWWVNGKEVHDGVCTDPQPLKEQPALNDSRYALSSRLRVSATFWQDPRNHFRCQVQFYGLSENDEWTQDRAKPVTQIVSAEAWGRADCGGGGSASERKSCVECPPCPAPEFEGGPSVFLFPPKPKDTLMISRTPEVTCVVVDVSQEDPEVQFNWYVDGVEVHNAKTKPREEQYNSTYRVVSVLTVLHQDWLNGKEYKCKVSNKALPASIEKTISKAKGQPREPQVCTLPPSQEEMTKNQVSLSCAVKGFYPSDIAVEWESNGQPENNYKTTPPVLDSDGSFFLVSKLTVDKSRWQEGNVFSCSVMHEALHNHYTQKSLSLSPGK

SEQ ID NO: 77 - protein, 10 aa, synthetic construct
ALSPTVWLSV

SEQ ID NO: 78 - protein, 10 aa, synthetic construct
GASPTVWLSV

SEQ ID NO: 79 - protein, 10 aa, synthetic construct
GLAPTVWLSV

SEQ ID NO: 80 - protein, 10 aa, synthetic construct
GLSATVWLSV

SEQ ID NO: 81 - protein, 10 aa, synthetic construct
GLSPAVWLSV

SEQ ID NO: 82 - protein, 10 aa, synthetic construct
GLSPVAWLSV

SEQ ID NO: 83 - protein, 10 aa, synthetic construct
GLSPTVALSV

SEQ ID NO: 84 - protein, 10 aa, synthetic construct
GLSPTVWASV

SEQ ID NO: 85 - protein, 10 aa, synthetic construct
GLSPTVWLAV

SEQ ID NO: 86 - protein, 10 aa, synthetic construct
GLSPTVWLSA

SEQ ID NO: 87 - protein, 9 aa, synthetic construct
FLLTRILTI

SEQ ID NO: 88 - protein, 160 aa, synthetic construct
EVQLVESGGGLVQPGGSLRLSCAASDDTYMTNCMGWFRQAPGKERVGVAAIYTGGGRAVYADSVRGRFTISQDNAKNTVYLQMNSLKPEDTAMYYCAADWLGPDMTDIQVLGALPWFNYWGQGTLVTVSSSAWSHPQFEKGGGSGGGSGGSAWSHPQFEK